European Patent Specification EP 3 885 357 B1, published January 1, 2025. Title: AN INTERLEUKIN 21 PROTEIN (IL21) MUTANT AND APPLICATION THEREOF. Applicant: HYQUO MOLECULE (BEIJING) TECHNOLOGY CO., LTD. The sequence listing filed with the application follows.

SEQUENCE LISTING (6 sequences)

SEQ ID NO: 1 - protein, 133 aa, Artificial Sequence [sequence omitted]

SEQ ID NO: 2 - protein, 127 aa, Artificial Sequence
QGQDRHMIRMRQLIDIVDQLKNYVNDLVPEFLPAPEDVETNCEWSAFSCFQKAQLKSANTGNNERIINVSIKKLKRNLWGLAGLNSCPSCDSYEKKPPKEFLERFKSLLQKMIHQHLSSRTHGSEDS

SEQ ID NO: 3 - protein, 133 aa, Artificial Sequence
QGQDRHMIRMRQLIDCVDQLKNYVNDLVPEFLPAPEDVETNCEWSAFSCFQKAQLKSANTGNNERIINVCIKKLKRKPPSTNAGRRQKHRLTCPSCDSYEKKPPKEFLERFKSLLQKMIHQHLSSRTHGSEDS

SEQ ID NO: 4 - protein, 127 aa, Artificial Sequence
QGQDRHMIRMRQLIDCVDQLKNYVNDLVPEFLPAPEDVETNCEWSAFSCFQKAQLKSANTGNNERIINVCIKKLKRNLWGLAGLNSCPSCDSYEKKPPKEFLERFKSLLQKMIHQHLSSRTHGSEDS

SEQ ID NO: 5 - protein, 133 aa, Artificial Sequence
QGQDRHMIRMRQLIDCCDQLKNYVNDLVPEFLPAPEDVETNCEWSAFSCFQKAQLKSANTGNNERIINVCIKKLKRKPPSTNAGRRQKHRLTCPSCDSYEKKPPKEFLERFCSLLQKMIHQHLSSRTHGSEDS

SEQ ID NO: 6 - protein, 127 aa, Artificial Sequence
QGQDRHMIRMRQLIDCCDQLKNYVNDLVPEFLPAPEDVETNCEWSAFSCFQKAQLKSANTGNNERIINVCIKKLKRNLWGLAGLNSCPSCDSYEKKPPKEFLERFCSLLQKMIHQHLSSRTHGSEDS